European Patent Application EP 4 471 159 A1, published December 4, 2024. Title: CRISPR nuclease off-target detection by sequencing (CROFT-Seq). Applicant: VILNIUS UNIVERSITY. Application EP. The sequence listing filed with the application follows.

SEQUENCE LISTING (11 sequences)

SEQ ID NO: 1 - RNA, 20 nt, synthetic construct
  source 1..20: mol_type = other RNA
ggaatcccttctgcagcacc

SEQ ID NO: 2 - RNA, 20 nt, synthetic construct
  source 1..20: mol_type = other RNA
gggtggggggagtttgctcc

SEQ ID NO: 3 - RNA, 20 nt, synthetic construct
  source 1..20: mol_type = other RNA
ggtggacaagcggcagatag

SEQ ID NO: 4 - DNA, 20 bp, synthetic construct
  source 1..20: mol_type = other DNA
acacgacgctcttccgatct

SEQ ID NO: 5 - DNA, 13 bp, synthetic construct
  source 1..13: mol_type = other DNA
agatcggaagagg

SEQ ID NO: 6 - DNA, 32 bp, synthetic construct
  source 1..32: mol_type = other DNA
cttggcacccgagaattccannnnnnnnnnnn

SEQ ID NO: 7 - DNA, 33 bp, synthetic construct
  source 1..33: mol_type = other DNA
cttggcacccgagaattccaggggggggggggh

SEQ ID NO: 8 - DNA, 62 bp, synthetic construct
  source 1..62: mol_type = other DNA
aatgatacggcgaccaccgagatctacacacactctttccctacacgacgctcttccgatct

SEQ ID NO: 9 - DNA, 57 bp, synthetic construct
  source 1..57: mol_type = other DNA
caagcagaagacggcatacgagatgtgactggagttccttggcacccgagaattcca

SEQ ID NO: 10 - DNA, 70 bp, synthetic construct
  source 1..70: mol_type = other DNA
aatgatacggcgaccaccgagatctacacnnnnnnnnacactctttccctacacgacgctcttccgatct

SEQ ID NO: 11 - DNA, 65 bp, synthetic construct
  source 1..65: mol_type = other DNA
caagcagaagacggcatacgagatnnnnnnnngtgactggagttccttggcacccgagaattcca